European Patent Application EP 4 628 508 A1, published October 8, 2025. Title: 抗ILT4抗体及其制备方法和应用. Applicant: 诺纳生物（苏州）有限公司. The sequence listing filed with the application follows.

SEQUENCE LISTING (138 sequences)

SEQ ID NO: 1 - protein, 10 aa, synthetic construct
GGSLSGYYWS

SEQ ID NO: 2 - protein, 16 aa, synthetic construct
EINHSGGTNYNPSLKS

SEQ ID NO: 3 - protein, 11 aa, synthetic construct
GQQQLDWYFDL

SEQ ID NO: 4 - protein, 11 aa, synthetic construct
RASQNIYSHLV

SEQ ID NO: 5 - protein, 7 aa, synthetic construct
GASTRAT

SEQ ID NO: 6 - protein, 10 aa, synthetic construct
QQYNDWPPIT

SEQ ID NO: 7 - protein, 16 aa, synthetic construct
EIQHSGGTNYNPSLKS

SEQ ID NO: 8 - protein, 16 aa, synthetic construct
EIAHSGGTNYNPSLKS

SEQ ID NO: 9 - protein, 16 aa, synthetic construct
EITHSGGTNYNPSLKS

SEQ ID NO: 10 - protein, 16 aa, synthetic construct
EINHAGGTNYNPSLKS

SEQ ID NO: 11 - protein, 16 aa, synthetic construct
EINHGGGTNYNPSLKS

SEQ ID NO: 12 - protein, 10 aa, synthetic construct
RFTFSTYAMS

SEQ ID NO: 13 - protein, 17 aa, synthetic construct
SISGSGFNTYYADSVKG

SEQ ID NO: 14 - protein, 11 aa, synthetic construct
DRQWLVSSFDY

SEQ ID NO: 15 - protein, 11 aa, synthetic construct
QASQDISNYLN

SEQ ID NO: 16 - protein, 7 aa, synthetic construct
DASNLET

SEQ ID NO: 17 - protein, 8 aa, synthetic construct
QQYDNLIT

SEQ ID NO: 18 - protein, 10 aa, synthetic construct
GDSISSYYWS

SEQ ID NO: 19 - protein, 16 aa, synthetic construct
FIYYSGSTNYNPSLKS

SEQ ID NO: 20 - protein, 11 aa, synthetic construct
QLWFGESPFDY

SEQ ID NO: 21 - protein, 11 aa, synthetic construct
RASQSVSSNLA

SEQ ID NO: 22 - protein, 9 aa, synthetic construct
QQYNNWPLT

SEQ ID NO: 23 - protein, 10 aa, synthetic construct
GFTFSSYAMS

SEQ ID NO: 24 - protein, 17 aa, synthetic construct
AISDNAGSTYYADSVKG

SEQ ID NO: 25 - protein, 12 aa, synthetic construct
ERQWLVLGVMDA

SEQ ID NO: 26 - protein, 9 aa, synthetic construct
QQNDNLPFT

SEQ ID NO: 27 - protein, 17 aa, synthetic construct
TISGSGGSAYYADSVKG

SEQ ID NO: 28 - protein, 9 aa, synthetic construct
LSGDDAFDI

SEQ ID NO: 29 - protein, 16 aa, synthetic construct
RSSQSLLRGNGYNYLD

SEQ ID NO: 30 - protein, 7 aa, synthetic construct
LGSNRAS

SEQ ID NO: 31 - protein, 9 aa, synthetic construct
MQALQSPLT

SEQ ID NO: 32 - protein, 10 aa, synthetic construct
GFTFSSYGMH

SEQ ID NO: 33 - protein, 17 aa, synthetic construct
GMWYDGNYKYYADSVKG

SEQ ID NO: 34 - protein, 9 aa, synthetic construct
DSPIGVFDY

SEQ ID NO: 35 - protein, 17 aa, synthetic construct
GMWYEGNYKYYADSVKG

SEQ ID NO: 36 - protein, 10 aa, synthetic construct
GFTFSTYAMT

SEQ ID NO: 37 - protein, 17 aa, synthetic construct
SISGSDFNTYYADSVKG

SEQ ID NO: 38 - protein, 11 aa, synthetic construct
DQEWLVRSFHH

SEQ ID NO: 39 - protein, 16 aa, synthetic construct
RSSQSLLRGNAYNYLD

SEQ ID NO: 40 - protein, 8 aa, synthetic construct
QQYENLPT

SEQ ID NO: 41 - protein, 17 aa, synthetic construct
TINHIGDSTYYADSVKG

SEQ ID NO: 42 - protein, 9 aa, synthetic construct
DQWFGVFDY

SEQ ID NO: 43 - protein, 8 aa, synthetic construct
QQYDNLPH

SEQ ID NO: 44 - protein, 10 aa, synthetic construct
GGSFSGYYWS

SEQ ID NO: 45 - protein, 16 aa, synthetic construct
EVSHSGGTNYNPSLKS

SEQ ID NO: 46 - protein, 13 aa, synthetic construct
SPYYGDYMYVFDI

SEQ ID NO: 47 - protein, 12 aa, synthetic construct
RASQSVSSSYLA

SEQ ID NO: 48 - protein, 7 aa, synthetic construct
GASSRAT

SEQ ID NO: 49 - protein, 8 aa, synthetic construct
QQYGSLFT

SEQ ID NO: 50 - protein, 17 aa, synthetic construct
SISGSDFSTYYADSVKG

SEQ ID NO: 51 - protein, 11 aa, synthetic construct
DRQWLVSSFDF

SEQ ID NO: 52 - protein, 11 aa, synthetic construct
GGSISSSNWWS

SEQ ID NO: 53 - protein, 16 aa, synthetic construct
EVYHSGSTNYNPSLKS

SEQ ID NO: 54 - protein, 14 aa, synthetic construct
VTGNKDYYYYDLDV

SEQ ID NO: 55 - protein, 7 aa, synthetic construct
DASNLGT

SEQ ID NO: 56 - protein, 9 aa, synthetic construct
QQYDNLPRT

SEQ ID NO: 57 - protein, 17 aa, synthetic construct
GIWYAGSNEYYVDSVKG

SEQ ID NO: 58 - protein, 9 aa, synthetic construct
DQGWGTMDA

SEQ ID NO: 59 - protein, 8 aa, synthetic construct
QQYDNLLT

SEQ ID NO: 60 - protein, 118 aa, synthetic construct
QVQLVESGGGVVQPGRSLRLSCAASGFTFSSYGMHWVRQAPGKGLGWVAGIWYAGSNEYYVDSVKGRFIISRDNSKNTLYLQMNSLRAEDTAVYYCARDQGWGTMDAWGQGASVTVSS

SEQ ID NO: 61 - protein, 119 aa, synthetic construct
QVQLQQWGAGLLKPSETLSLTCAVYGGSLSGYYWSWIRQPPGKGLEWIGEINHSGGTNYNPSLKSRVTISVPTSKNQFSLKLTSVTAADTAVYYCARGQQQLDWYFDLWGRGTLVTVSS

SEQ ID NO: 62 - protein, 108 aa, synthetic construct
EIVMTQSPATLSVSPGERATLSCRASQNIYSHLVWYQQKPGQAPRLLIYGASTRATGIPARFSGSGSGTEFTLTITSLQSEDFTVYYCQQYNDWPPITFGQGTRLEIR

SEQ ID NO: 63 - protein, 119 aa, synthetic construct
QVQLQQWGAGLLKPSETLSLTCAVYGGSLSGYYWSWIRQPPGKGLEWIGEIQHSGGTNYNPSLKSRVTISVPTSKNQFSLKLTSVTAADTAVYYCARGQQQLDWYFDLWGRGTLVTVSS

SEQ ID NO: 64 - protein, 119 aa, synthetic construct
QVQLQQWGAGLLKPSETLSLTCAVYGGSLSGYYWSWIRQPPGKGLEWIGEIAHSGGTNYNPSLKSRVTISVPTSKNQFSLKLTSVTAADTAVYYCARGQQQLDWYFDLWGRGTLVTVSS

SEQ ID NO: 65 - protein, 119 aa, synthetic construct
QVQLQQWGAGLLKPSETLSLTCAVYGGSLSGYYWSWIRQPPGKGLEWIGEITHSGGTNYNPSLKSRVTISVPTSKNQFSLKLTSVTAADTAVYYCARGQQQLDWYFDLWGRGTLVTVSS

SEQ ID NO: 66 - protein, 119 aa, synthetic construct
QVQLQQWGAGLLKPSETLSLTCAVYGGSLSGYYWSWIRQPPGKGLEWIGEINHAGGTNYNPSLKSRVTISVPTSKNQFSLKLTSVTAADTAVYYCARGQQQLDWYFDLWGRGTLVTVSS

SEQ ID NO: 67 - protein, 119 aa, synthetic construct
QVQLQQWGAGLLKPSETLSLTCAVYGGSLSGYYWSWIRQPPGKGLEWIGEINHGGGTNYNPSLKSRVTISVPTSKNQFSLKLTSVTAADTAVYYCARGQQQLDWYFDLWGRGTLVTVSS

SEQ ID NO: 68 - protein, 120 aa, synthetic construct
EVQLLESGGGLVQPGGSLRLSCAASRFTFSTYAMSWVRQAPGKGLEWVSSISGSGFNTYYADSVKGRFTISSDSSKNTLYLQMNSLRAEDTAVYYCAKDRQWLVSSFDYWGQGTLVTVSS

SEQ ID NO: 69 - protein, 106 aa, synthetic construct
DIQMTQSPSSLSASVGDRVTITCQASQDISNYLNWYQQKPGKAPKLLIYDASNLETGVPSRFSGSGSGTDFTFTISSLQPEDIATYYCQQYDNLITFGQGTRLEIK

SEQ ID NO: 70 - protein, 119 aa, synthetic construct
QVQLQESGPGLVKPSETLSLTCTVSGDSISSYYWSWIRQPPGKGLEWIGFIYYSGSTNYNPSLKSRVTISVDTSKNQFSLKLTSVTAADTAVYYCANQLWFGESPFDYWGQGTLVTVSS

SEQ ID NO: 71 - protein, 107 aa, synthetic construct
EIVMTQSPATLSVSPGERATLSCRASQSVSSNLAWYQQKPGQAPRLLIYGASTRATGIPARFSGSGSGTEFTLTISSLQSEDFAVYYCQQYNNWPLTFGGGTKVEIK

SEQ ID NO: 72 - protein, 121 aa, synthetic construct
EVQLLESGGGLVQPGGSLRLSCAVSGFTFSSYAMSWVRQAPGKGLEWVSAISDNAGSTYYADSVKGRFTISRDNSKNTLHLQMNSLRAEDTAVYSCAKERQWLVLGVMDAWGQGASVTVSS

SEQ ID NO: 73 - protein, 107 aa, synthetic construct
DIQMTQSPSSLSASVGDRVTITCQASQDISNYLNWYQQKPGKARKLLISDASNLETGVPSRFSGSGSGTDFTFTISSLEPEDIATYHCQQNDNLPFTFGPGTKVEIK

SEQ ID NO: 74 - protein, 118 aa, synthetic construct
EVQLLESGGGLVQSGGSLRLSCAASGFTFSSYAMSWVRQAPGKGLGWVSTISGSGGSAYYADSVKGRFTVSRDNSKKTLYLQMNSLRAEDTAVYFCAILSGDDAFDIWGQGTMVTVSS

SEQ ID NO: 75 - protein, 112 aa, synthetic construct
DVVMTQSPLSLPVTPGEPASISCRSSQSLLRGNGYNYLDWYLQKPGQSPQLLIYLGSNRASGVPDRFSGSGSGTDFTLKISRVEAEDVGIFYCMQALQSPLTFGGGTKVEIK

SEQ ID NO: 76 - protein, 112 aa, synthetic construct
DVVMTQSPLSLPVTPGEPASISCRSSQSLLRGNAYNYLDWYLQKPGQSPQLLIYLGSNRASGVPDRFSGSGSGTDFTLKISRVEAEDVGIFYCMQALQSPLTFGGGTKVEIK

SEQ ID NO: 77 - protein, 118 aa, synthetic construct
QVQLVESGGTVVQSGRSLRLSCAASGFTFSSYGMHWVRQAPGKGLEWVAGMWYDGNYKYYADSVKGRFTISRDNSKNTLSLQMNSLRAEDTAVYYCARDSPIGVFDYWGQGTLVTVSS

SEQ ID NO: 78 - protein, 106 aa, synthetic construct; identical to SEQ ID NO: 69

SEQ ID NO: 79 - protein, 118 aa, synthetic construct
QVQLVESGGTVVQSGRSLRLSCAASGFTFSSYGMHWVRQAPGKGLEWVAGMWYEGNYKYYADSVKGRFTISRDNSKNTLSLQMNSLRAEDTAVYYCARDSPIGVFDYWGQGTLVTVSS

SEQ ID NO: 80 - protein, 120 aa, synthetic construct
EVQLLESGGGLVQPGGSLRLSCAASGFTFSTYAMTWVRQAPGKGLEWVSSISGSDFNTYYADSVKGRFTISRDISKNTLYLQMNSLRAEDTAVYYCAKDQEWLVRSFHHWGQGTLVTVSS

SEQ ID NO: 81 - protein, 106 aa, synthetic construct
DIQMTQFPSSLFAFVGDRVTITCQASQDISNYLNWYQQKAGKAPKLLINDASNLETGVPSRFSGSGFGTDFTFTISSLQPEDFATYYCQQYENLPTFGGGTKVEIK

SEQ ID NO: 82 - protein, 118 aa, synthetic construct
EVQLLESGGGLVQPGGSLRLSCAASGFTFSSYAMSWVRQAPGKGLEWVSTINHIGDSTYYADSVKGRFTISRDNSKNTLYLQMNSLRAEDTAVYYCAKDQWFGVFDYWGQGTLVTVSS

SEQ ID NO: 83 - protein, 106 aa, synthetic construct
DIQMTQSPSSLSASVGDRVTITCQASQDISNYLNWYQQKPGKAPKLLIYDASNLETGVPSRFSGSGSGTDFTFTISSLQPEDIATYYCQQYDNLPHFGQGTKLEIK

SEQ ID NO: 84 - protein, 121 aa, synthetic construct
QVQLQQWGAGLLKPSETLSLTCAVYGGSFSGYYWSWIRQTLGKGLEWIGEVSHSGGTNYNPSLKSRVTISVDTSKNQFSLKLSSVTAADTAVYYCARSPYYGDYMYVFDIWGQGTMVTVSS

SEQ ID NO: 85 - protein, 107 aa, synthetic construct
EIVLTQSPGTLSLSPGERATLSCRASQSVSSSYLAWYQQKPGQAPRLLIYGASSRATGIPDRFSGSGSGTDFTLTISRLEPEDFAVYYCQQYGSLFTFGGGTKVEIK

SEQ ID NO: 86 - protein, 120 aa, synthetic construct
EVQLLESGGGLVQPGGSLRLSCAASGFTFSSYAMSWVRQAPGKGLEWVSSISGSDFSTYYADSVKGRFTISRDTSKNTLYLQMNSLRAEDTAVYYCAKDRQWLVSSFDFWGQGALVTVSS

SEQ ID NO: 87 - protein, 123 aa, synthetic construct
QVQLQESGPGLVKPSGTLSLTCAVSGGSISSSNWWSWVRQPPGKGLEWIGEVYHSGSTNYNPSLKSRVTISVDKSQNQFSLKLTSVTAADTAVYYCARVTGNKDYYYYDLDVWGQGTTVTVSS

SEQ ID NO: 88 - protein, 107 aa, synthetic construct
DIQMTQSPSSLSASVGDRVTITCQASQDISNYLNWYQQKPGKAPKLLIYDASNLGTGVPSRFSGGGSGTDFTFTISSLQPEDIATYYCQQYDNLPRTFGQGTKVEIK

SEQ ID NO: 89 - protein, 106 aa, synthetic construct
DIQMTQSPSSLSASVGDRVTITCQASQDISNYLNWYQQKPGKAPKLLIYDASNLETGVPSRFSGSGSGTDFTFTISSLQPEDIAIYYCQQYDNLLTFGGGTKVEIK

SEQ ID NO: 90 - protein, 449 aa, synthetic construct
QVQLQQWGAGLLKPSETLSLTCAVYGGSLSGYYWSWIRQPPGKGLEWIGEINHSGGTNYNPSLKSRVTISVPTSKNQFSLKLTSVTAADTAVYYCARGQQQLDWYFDLWGRGTLVTVSSASTKGPSVFPLAPSSKSTSGGTAALGCLVKDYFPEPVTVSWNSGALTSGVHTFPAVLQSSGLYSLSSVVTVPSSSLGTQTYICNVNHKPSNTKVDKKVEPKSCDKTHTCPPCPAPELLGGPSVFLFPPKPKDTLMISRTPEVTCVVVDVSHEDPEVKFNWYVDGVEVHNAKTKPREEQYNSTYRVVSVLTVLHQDWLNGKEYKCKVSNKALPAPIEKTISKAKGQPREPQVYTLPPSREEMTKNQVSLTCLVKGFYPSDIAVEWESNGQPENNYKTTPPVLDSDGSFFLYSKLTVDKSRWQQGNVFSCSVMHEALHNHYTQKSLSLSPGK

SEQ ID NO: 91 - protein, 215 aa, synthetic construct
EIVMTQSPATLSVSPGERATLSCRASQNIYSHLVWYQQKPGQAPRLLIYGASTRATGIPARFSGSGSGTEFTLTITSLQSEDFTVYYCQQYNDWPPITFGQGTRLEIRRTVAAPSVFIFPPSDEQLKSGTASVVCLLNNFYPREAKVQWKVDNALQSGNSQESVTEQDSKDSTYSLSSTLTLSKADYEKHKVYACEVTHQGLSSPVTKSFNRGEC

SEQ ID NO: 92 - protein, 446 aa, synthetic construct
QVQLQQWGAGLLKPSETLSLTCAVYGGSLSGYYWSWIRQPPGKGLEWIGEIQHSGGTNYNPSLKSRVTISVPTSKNQFSLKLTSVTAADTAVYYCARGQQQLDWYFDLWGRGTLVTVSSASTKGPSVFPLAPCSRSTSESTAALGCLVKDYFPEPVTVSWNSGALTSGVHTFPAVLQSSGLYSLSSVVTVPSSSLGTKTYTCNVDHKPSNTKVDKRVESKYGPPCPPCPAPEFLGGPSVFLFPPKPKDTLMISRTPEVTCVVVDVSQEDPEVQFNWYVDGVEVHNAKTKPREEQFNSTYRVVSVLTVLHQDWLNGKEYKCKVSNKGLPSSIEKTISKAKGQPREPQVYTLPPSQEEMTKNQVSLTCLVKGFYPSDIAVEWESNGQPENNYKTTPPVLDSDGSFFLYSRLTVDKSRWQEGNVFSCSVMHEALHNHYTQKSLSLSLGK

SEQ ID NO: 93 - protein, 446 aa, synthetic construct
QVQLQQWGAGLLKPSETLSLTCAVYGGSLSGYYWSWIRQPPGKGLEWIGEIAHSGGTNYNPSLKSRVTISVPTSKNQFSLKLTSVTAADTAVYYCARGQQQLDWYFDLWGRGTLVTVSSASTKGPSVFPLAPCSRSTSESTAALGCLVKDYFPEPVTVSWNSGALTSGVHTFPAVLQSSGLYSLSSVVTVPSSSLGTKTYTCNVDHKPSNTKVDKRVESKYGPPCPPCPAPEFLGGPSVFLFPPKPKDTLMISRTPEVTCVVVDVSQEDPEVQFNWYVDGVEVHNAKTKPREEQFNSTYRVVSVLTVLHQDWLNGKEYKCKVSNKGLPSSIEKTISKAKGQPREPQVYTLPPSQEEMTKNQVSLTCLVKGFYPSDIAVEWESNGQPENNYKTTPPVLDSDGSFFLYSRLTVDKSRWQEGNVFSCSVMHEALHNHYTQKSLSLSLGK

SEQ ID NO: 94 - protein, 446 aa, synthetic construct
QVQLQQWGAGLLKPSETLSLTCAVYGGSLSGYYWSWIRQPPGKGLEWIGEITHSGGTNYNPSLKSRVTISVPTSKNQFSLKLTSVTAADTAVYYCARGQQQLDWYFDLWGRGTLVTVSSASTKGPSVFPLAPCSRSTSESTAALGCLVKDYFPEPVTVSWNSGALTSGVHTFPAVLQSSGLYSLSSVVTVPSSSLGTKTYTCNVDHKPSNTKVDKRVESKYGPPCPPCPAPEFLGGPSVFLFPPKPKDTLMISRTPEVTCVVVDVSQEDPEVQFNWYVDGVEVHNAKTKPREEQFNSTYRVVSVLTVLHQDWLNGKEYKCKVSNKGLPSSIEKTISKAKGQPREPQVYTLPPSQEEMTKNQVSLTCLVKGFYPSDIAVEWESNGQPENNYKTTPPVLDSDGSFFLYSRLTVDKSRWQEGNVFSCSVMHEALHNHYTQKSLSLSLGK

SEQ ID NO: 95 - protein, 446 aa, synthetic construct
QVQLQQWGAGLLKPSETLSLTCAVYGGSLSGYYWSWIRQPPGKGLEWIGEINHAGGTNYNPSLKSRVTISVPTSKNQFSLKLTSVTAADTAVYYCARGQQQLDWYFDLWGRGTLVTVSSASTKGPSVFPLAPCSRSTSESTAALGCLVKDYFPEPVTVSWNSGALTSGVHTFPAVLQSSGLYSLSSVVTVPSSSLGTKTYTCNVDHKPSNTKVDKRVESKYGPPCPPCPAPEFLGGPSVFLFPPKPKDTLMISRTPEVTCVVVDVSQEDPEVQFNWYVDGVEVHNAKTKPREEQFNSTYRVVSVLTVLHQDWLNGKEYKCKVSNKGLPSSIEKTISKAKGQPREPQVYTLPPSQEEMTKNQVSLTCLVKGFYPSDIAVEWESNGQPENNYKTTPPVLDSDGSFFLYSRLTVDKSRWQEGNVFSCSVMHEALHNHYTQKSLSLSLGK

SEQ ID NO: 96 - protein, 446 aa, synthetic construct
QVQLQQWGAGLLKPSETLSLTCAVYGGSLSGYYWSWIRQPPGKGLEWIGEINHGGGTNYNPSLKSRVTISVPTSKNQFSLKLTSVTAADTAVYYCARGQQQLDWYFDLWGRGTLVTVSSASTKGPSVFPLAPCSRSTSESTAALGCLVKDYFPEPVTVSWNSGALTSGVHTFPAVLQSSGLYSLSSVVTVPSSSLGTKTYTCNVDHKPSNTKVDKRVESKYGPPCPPCPAPEFLGGPSVFLFPPKPKDTLMISRTPEVTCVVVDVSQEDPEVQFNWYVDGVEVHNAKTKPREEQFNSTYRVVSVLTVLHQDWLNGKEYKCKVSNKGLPSSIEKTISKAKGQPREPQVYTLPPSQEEMTKNQVSLTCLVKGFYPSDIAVEWESNGQPENNYKTTPPVLDSDGSFFLYSRLTVDKSRWQEGNVFSCSVMHEALHNHYTQKSLSLSLGK

SEQ ID NO: 97 - protein, 450 aa, synthetic construct
EVQLLESGGGLVQPGGSLRLSCAASRFTFSTYAMSWVRQAPGKGLEWVSSISGSGFNTYYADSVKGRFTISSDSSKNTLYLQMNSLRAEDTAVYYCAKDRQWLVSSFDYWGQGTLVTVSSASTKGPSVFPLAPSSKSTSGGTAALGCLVKDYFPEPVTVSWNSGALTSGVHTFPAVLQSSGLYSLSSVVTVPSSSLGTQTYICNVNHKPSNTKVDKKVEPKSCDKTHTCPPCPAPELLGGPSVFLFPPKPKDTLMISRTPEVTCVVVDVSHEDPEVKFNWYVDGVEVHNAKTKPREEQYNSTYRVVSVLTVLHQDWLNGKEYKCKVSNKALPAPIEKTISKAKGQPREPQVYTLPPSREEMTKNQVSLTCLVKGFYPSDIAVEWESNGQPENNYKTTPPVLDSDGSFFLYSKLTVDKSRWQQGNVFSCSVMHEALHNHYTQKSLSLSPGK

SEQ ID NO: 98 - protein, 213 aa, synthetic construct
DIQMTQSPSSLSASVGDRVTITCQASQDISNYLNWYQQKPGKAPKLLIYDASNLETGVPSRFSGSGSGTDFTFTISSLQPEDIATYYCQQYDNLITFGQGTRLEIKRTVAAPSVFIFPPSDEQLKSGTASVVCLLNNFYPREAKVQWKVDNALQSGNSQESVTEQDSKDSTYSLSSTLTLSKADYEKHKVYACEVTHQGLSSPVTKSFNRGEC

SEQ ID NO: 99 - protein, 447 aa, synthetic construct
EVQLLESGGGLVQPGGSLRLSCAASRFTFSTYAMSWVRQAPGKGLEWVSSISGSGFNTYYADSVKGRFTISSDSSKNTLYLQMNSLRAEDTAVYYCAKDRQWLVSSFDYWGQGTLVTVSSASTKGPSVFPLAPCSRSTSESTAALGCLVKDYFPEPVTVSWNSGALTSGVHTFPAVLQSSGLYSLSSVVTVPSSSLGTKTYTCNVDHKPSNTKVDKRVESKYGPPCPPCPAPEFLGGPSVFLFPPKPKDTLMISRTPEVTCVVVDVSQEDPEVQFNWYVDGVEVHNAKTKPREEQFNSTYRVVSVLTVLHQDWLNGKEYKCKVSNKGLPSSIEKTISKAKGQPREPQVYTLPPSQEEMTKNQVSLTCLVKGFYPSDIAVEWESNGQPENNYKTTPPVLDSDGSFFLYSRLTVDKSRWQEGNVFSCSVMHEALHNHYTQKSLSLSLGK

SEQ ID NO: 100 - protein, 449 aa, synthetic construct
QVQLQESGPGLVKPSETLSLTCTVSGDSISSYYWSWIRQPPGKGLEWIGFIYYSGSTNYNPSLKSRVTISVDTSKNQFSLKLTSVTAADTAVYYCANQLWFGESPFDYWGQGTLVTVSSASTKGPSVFPLAPSSKSTSGGTAALGCLVKDYFPEPVTVSWNSGALTSGVHTFPAVLQSSGLYSLSSVVTVPSSSLGTQTYICNVNHKPSNTKVDKKVEPKSCDKTHTCPPCPAPELLGGPSVFLFPPKPKDTLMISRTPEVTCVVVDVSHEDPEVKFNWYVDGVEVHNAKTKPREEQYNSTYRVVSVLTVLHQDWLNGKEYKCKVSNKALPAPIEKTISKAKGQPREPQVYTLPPSREEMTKNQVSLTCLVKGFYPSDIAVEWESNGQPENNYKTTPPVLDSDGSFFLYSKLTVDKSRWQQGNVFSCSVMHEALHNHYTQKSLSLSPGK

SEQ ID NO: 101 - protein, 214 aa, synthetic construct
EIVMTQSPATLSVSPGERATLSCRASQSVSSNLAWYQQKPGQAPRLLIYGASTRATGIPARFSGSGSGTEFTLTISSLQSEDFAVYYCQQYNNWPLTFGGGTKVEIKRTVAAPSVFIFPPSDEQLKSGTASVVCLLNNFYPREAKVQWKVDNALQSGNSQESVTEQDSKDSTYSLSSTLTLSKADYEKHKVYACEVTHQGLSSPVTKSFNRGEC

SEQ ID NO: 102 - protein, 446 aa, synthetic construct
QVQLQESGPGLVKPSETLSLTCTVSGDSISSYYWSWIRQPPGKGLEWIGFIYYSGSTNYNPSLKSRVTISVDTSKNQFSLKLTSVTAADTAVYYCANQLWFGESPFDYWGQGTLVTVSSASTKGPSVFPLAPCSRSTSESTAALGCLVKDYFPEPVTVSWNSGALTSGVHTFPAVLQSSGLYSLSSVVTVPSSSLGTKTYTCNVDHKPSNTKVDKRVESKYGPPCPPCPAPEFLGGPSVFLFPPKPKDTLMISRTPEVTCVVVDVSQEDPEVQFNWYVDGVEVHNAKTKPREEQFNSTYRVVSVLTVLHQDWLNGKEYKCKVSNKGLPSSIEKTISKAKGQPREPQVYTLPPSQEEMTKNQVSLTCLVKGFYPSDIAVEWESNGQPENNYKTTPPVLDSDGSFFLYSRLTVDKSRWQEGNVFSCSVMHEALHNHYTQKSLSLSLGK

SEQ ID NO: 103 - protein, 451 aa, synthetic construct
EVQLLESGGGLVQPGGSLRLSCAVSGFTFSSYAMSWVRQAPGKGLEWVSAISDNAGSTYYADSVKGRFTISRDNSKNTLHLQMNSLRAEDTAVYSCAKERQWLVLGVMDAWGQGASVTVSSASTKGPSVFPLAPSSKSTSGGTAALGCLVKDYFPEPVTVSWNSGALTSGVHTFPAVLQSSGLYSLSSVVTVPSSSLGTQTYICNVNHKPSNTKVDKKVEPKSCDKTHTCPPCPAPELLGGPSVFLFPPKPKDTLMISRTPEVTCVVVDVSHEDPEVKFNWYVDGVEVHNAKTKPREEQYNSTYRVVSVLTVLHQDWLNGKEYKCKVSNKALPAPIEKTISKAKGQPREPQVYTLPPSREEMTKNQVSLTCLVKGFYPSDIAVEWESNGQPENNYKTTPPVLDSDGSFFLYSKLTVDKSRWQQGNVFSCSVMHEALHNHYTQKSLSLSPGK

SEQ ID NO: 104 - protein, 214 aa, synthetic construct
DIQMTQSPSSLSASVGDRVTITCQASQDISNYLNWYQQKPGKARKLLISDASNLETGVPSRFSGSGSGTDFTFTISSLEPEDIATYHCQQNDNLPFTFGPGTKVEIKRTVAAPSVFIFPPSDEQLKSGTASVVCLLNNFYPREAKVQWKVDNALQSGNSQESVTEQDSKDSTYSLSSTLTLSKADYEKHKVYACEVTHQGLSSPVTKSFNRGEC

SEQ ID NO: 105 - protein, 448 aa, synthetic construct
EVQLLESGGGLVQPGGSLRLSCAVSGFTFSSYAMSWVRQAPGKGLEWVSAISDNAGSTYYADSVKGRFTISRDNSKNTLHLQMNSLRAEDTAVYSCAKERQWLVLGVMDAWGQGASVTVSSASTKGPSVFPLAPCSRSTSESTAALGCLVKDYFPEPVTVSWNSGALTSGVHTFPAVLQSSGLYSLSSVVTVPSSSLGTKTYTCNVDHKPSNTKVDKRVESKYGPPCPPCPAPEFLGGPSVFLFPPKPKDTLMISRTPEVTCVVVDVSQEDPEVQFNWYVDGVEVHNAKTKPREEQFNSTYRVVSVLTVLHQDWLNGKEYKCKVSNKGLPSSIEKTISKAKGQPREPQVYTLPPSQEEMTKNQVSLTCLVKGFYPSDIAVEWESNGQPENNYKTTPPVLDSDGSFFLYSRLTVDKSRWQEGNVFSCSVMHEALHNHYTQKSLSLSLGK

SEQ ID NO: 106 - protein, 448 aa, synthetic construct
EVQLLESGGGLVQSGGSLRLSCAASGFTFSSYAMSWVRQAPGKGLGWVSTISGSGGSAYYADSVKGRFTVSRDNSKKTLYLQMNSLRAEDTAVYFCAILSGDDAFDIWGQGTMVTVSSASTKGPSVFPLAPSSKSTSGGTAALGCLVKDYFPEPVTVSWNSGALTSGVHTFPAVLQSSGLYSLSSVVTVPSSSLGTQTYICNVNHKPSNTKVDKKVEPKSCDKTHTCPPCPAPELLGGPSVFLFPPKPKDTLMISRTPEVTCVVVDVSHEDPEVKFNWYVDGVEVHNAKTKPREEQYNSTYRVVSVLTVLHQDWLNGKEYKCKVSNKALPAPIEKTISKAKGQPREPQVYTLPPSREEMTKNQVSLTCLVKGFYPSDIAVEWESNGQPENNYKTTPPVLDSDGSFFLYSKLTVDKSRWQQGNVFSCSVMHEALHNHYTQKSLSLSPGK

SEQ ID NO: 107 - protein, 219 aa, synthetic construct
DVVMTQSPLSLPVTPGEPASISCRSSQSLLRGNGYNYLDWYLQKPGQSPQLLIYLGSNRASGVPDRFSGSGSGTDFTLKISRVEAEDVGIFYCMQALQSPLTFGGGTKVEIKRTVAAPSVFIFPPSDEQLKSGTASVVCLLNNFYPREAKVQWKVDNALQSGNSQESVTEQDSKDSTYSLSSTLTLSKADYEKHKVYACEVTHQGLSSPVTKSFNRGEC

SEQ ID NO: 108 - protein, 445 aa, synthetic construct
EVQLLESGGGLVQSGGSLRLSCAASGFTFSSYAMSWVRQAPGKGLGWVSTISGSGGSAYYADSVKGRFTVSRDNSKKTLYLQMNSLRAEDTAVYFCAILSGDDAFDIWGQGTMVTVSSASTKGPSVFPLAPCSRSTSESTAALGCLVKDYFPEPVTVSWNSGALTSGVHTFPAVLQSSGLYSLSSVVTVPSSSLGTKTYTCNVDHKPSNTKVDKRVESKYGPPCPPCPAPEFLGGPSVFLFPPKPKDTLMISRTPEVTCVVVDVSQEDPEVQFNWYVDGVEVHNAKTKPREEQFNSTYRVVSVLTVLHQDWLNGKEYKCKVSNKGLPSSIEKTISKAKGQPREPQVYTLPPSQEEMTKNQVSLTCLVKGFYPSDIAVEWESNGQPENNYKTTPPVLDSDGSFFLYSRLTVDKSRWQEGNVFSCSVMHEALHNHYTQKSLSLSLGK

SEQ ID NO: 109 - protein, 219 aa, synthetic construct
DVVMTQSPLSLPVTPGEPASISCRSSQSLLRGNAYNYLDWYLQKPGQSPQLLIYLGSNRASGVPDRFSGSGSGTDFTLKISRVEAEDVGIFYCMQALQSPLTFGGGTKVEIKRTVAAPSVFIFPPSDEQLKSGTASVVCLLNNFYPREAKVQWKVDNALQSGNSQESVTEQDSKDSTYSLSSTLTLSKADYEKHKVYACEVTHQGLSSPVTKSFNRGEC

SEQ ID NO: 110 - protein, 448 aa, synthetic construct
QVQLVESGGTVVQSGRSLRLSCAASGFTFSSYGMHWVRQAPGKGLEWVAGMWYDGNYKYYADSVKGRFTISRDNSKNTLSLQMNSLRAEDTAVYYCARDSPIGVFDYWGQGTLVTVSSASTKGPSVFPLAPSSKSTSGGTAALGCLVKDYFPEPVTVSWNSGALTSGVHTFPAVLQSSGLYSLSSVVTVPSSSLGTQTYICNVNHKPSNTKVDKKVEPKSCDKTHTCPPCPAPELLGGPSVFLFPPKPKDTLMISRTPEVTCVVVDVSHEDPEVKFNWYVDGVEVHNAKTKPREEQYNSTYRVVSVLTVLHQDWLNGKEYKCKVSNKALPAPIEKTISKAKGQPREPQVYTLPPSREEMTKNQVSLTCLVKGFYPSDIAVEWESNGQPENNYKTTPPVLDSDGSFFLYSKLTVDKSRWQQGNVFSCSVMHEALHNHYTQKSLSLSPGK

SEQ ID NO: 111 - protein, 445 aa, synthetic construct
QVQLVESGGTVVQSGRSLRLSCAASGFTFSSYGMHWVRQAPGKGLEWVAGMWYDGNYKYYADSVKGRFTISRDNSKNTLSLQMNSLRAEDTAVYYCARDSPIGVFDYWGQGTLVTVSSASTKGPSVFPLAPCSRSTSESTAALGCLVKDYFPEPVTVSWNSGALTSGVHTFPAVLQSSGLYSLSSVVTVPSSSLGTKTYTCNVDHKPSNTKVDKRVESKYGPPCPPCPAPEFLGGPSVFLFPPKPKDTLMISRTPEVTCVVVDVSQEDPEVQFNWYVDGVEVHNAKTKPREEQFNSTYRVVSVLTVLHQDWLNGKEYKCKVSNKGLPSSIEKTISKAKGQPREPQVYTLPPSQEEMTKNQVSLTCLVKGFYPSDIAVEWESNGQPENNYKTTPPVLDSDGSFFLYSRLTVDKSRWQEGNVFSCSVMHEALHNHYTQKSLSLSLGK

SEQ ID NO: 112 - protein, 445 aa, synthetic construct
QVQLVESGGTVVQSGRSLRLSCAASGFTFSSYGMHWVRQAPGKGLEWVAGMWYEGNYKYYADSVKGRFTISRDNSKNTLSLQMNSLRAEDTAVYYCARDSPIGVFDYWGQGTLVTVSSASTKGPSVFPLAPCSRSTSESTAALGCLVKDYFPEPVTVSWNSGALTSGVHTFPAVLQSSGLYSLSSVVTVPSSSLGTKTYTCNVDHKPSNTKVDKRVESKYGPPCPPCPAPEFLGGPSVFLFPPKPKDTLMISRTPEVTCVVVDVSQEDPEVQFNWYVDGVEVHNAKTKPREEQFNSTYRVVSVLTVLHQDWLNGKEYKCKVSNKGLPSSIEKTISKAKGQPREPQVYTLPPSQEEMTKNQVSLTCLVKGFYPSDIAVEWESNGQPENNYKTTPPVLDSDGSFFLYSRLTVDKSRWQEGNVFSCSVMHEALHNHYTQKSLSLSLGK

SEQ ID NO: 113 - protein, 450 aa, synthetic construct
EVQLLESGGGLVQPGGSLRLSCAASGFTFSTYAMTWVRQAPGKGLEWVSSISGSDFNTYYADSVKGRFTISRDISKNTLYLQMNSLRAEDTAVYYCAKDQEWLVRSFHHWGQGTLVTVSSASTKGPSVFPLAPSSKSTSGGTAALGCLVKDYFPEPVTVSWNSGALTSGVHTFPAVLQSSGLYSLSSVVTVPSSSLGTQTYICNVNHKPSNTKVDKKVEPKSCDKTHTCPPCPAPELLGGPSVFLFPPKPKDTLMISRTPEVTCVVVDVSHEDPEVKFNWYVDGVEVHNAKTKPREEQYNSTYRVVSVLTVLHQDWLNGKEYKCKVSNKALPAPIEKTISKAKGQPREPQVYTLPPSREEMTKNQVSLTCLVKGFYPSDIAVEWESNGQPENNYKTTPPVLDSDGSFFLYSKLTVDKSRWQQGNVFSCSVMHEALHNHYTQKSLSLSPGK

SEQ ID NO: 114 - protein, 213 aa, synthetic construct
DIQMTQFPSSLFAFVGDRVTITCQASQDISNYLNWYQQKAGKAPKLLINDASNLETGVPSRFSGSGFGTDFTFTISSLQPEDFATYYCQQYENLPTFGGGTKVEIKRTVAAPSVFIFPPSDEQLKSGTASVVCLLNNFYPREAKVQWKVDNALQSGNSQESVTEQDSKDSTYSLSSTLTLSKADYEKHKVYACEVTHQGLSSPVTKSFNRGEC

SEQ ID NO: 115 - protein, 448 aa, synthetic construct
EVQLLESGGGLVQPGGSLRLSCAASGFTFSSYAMSWVRQAPGKGLEWVSTINHIGDSTYYADSVKGRFTISRDNSKNTLYLQMNSLRAEDTAVYYCAKDQWFGVFDYWGQGTLVTVSSASTKGPSVFPLAPSSKSTSGGTAALGCLVKDYFPEPVTVSWNSGALTSGVHTFPAVLQSSGLYSLSSVVTVPSSSLGTQTYICNVNHKPSNTKVDKKVEPKSCDKTHTCPPCPAPELLGGPSVFLFPPKPKDTLMISRTPEVTCVVVDVSHEDPEVKFNWYVDGVEVHNAKTKPREEQYNSTYRVVSVLTVLHQDWLNGKEYKCKVSNKALPAPIEKTISKAKGQPREPQVYTLPPSREEMTKNQVSLTCLVKGFYPSDIAVEWESNGQPENNYKTTPPVLDSDGSFFLYSKLTVDKSRWQQGNVFSCSVMHEALHNHYTQKSLSLSPGK

SEQ ID NO: 116 - protein, 213 aa, synthetic construct
DIQMTQSPSSLSASVGDRVTITCQASQDISNYLNWYQQKPGKAPKLLIYDASNLETGVPSRFSGSGSGTDFTFTISSLQPEDIATYYCQQYDNLPHFGQGTKLEIKRTVAAPSVFIFPPSDEQLKSGTASVVCLLNNFYPREAKVQWKVDNALQSGNSQESVTEQDSKDSTYSLSSTLTLSKADYEKHKVYACEVTHQGLSSPVTKSFNRGEC

SEQ ID NO: 117 - protein, 451 aa, synthetic construct
QVQLQQWGAGLLKPSETLSLTCAVYGGSFSGYYWSWIRQTLGKGLEWIGEVSHSGGTNYNPSLKSRVTISVDTSKNQFSLKLSSVTAADTAVYYCARSPYYGDYMYVFDIWGQGTMVTVSSASTKGPSVFPLAPSSKSTSGGTAALGCLVKDYFPEPVTVSWNSGALTSGVHTFPAVLQSSGLYSLSSVVTVPSSSLGTQTYICNVNHKPSNTKVDKKVEPKSCDKTHTCPPCPAPELLGGPSVFLFPPKPKDTLMISRTPEVTCVVVDVSHEDPEVKFNWYVDGVEVHNAKTKPREEQYNSTYRVVSVLTVLHQDWLNGKEYKCKVSNKALPAPIEKTISKAKGQPREPQVYTLPPSREEMTKNQVSLTCLVKGFYPSDIAVEWESNGQPENNYKTTPPVLDSDGSFFLYSKLTVDKSRWQQGNVFSCSVMHEALHNHYTQKSLSLSPGK

SEQ ID NO: 118 - protein, 214 aa, synthetic construct
EIVLTQSPGTLSLSPGERATLSCRASQSVSSSYLAWYQQKPGQAPRLLIYGASSRATGIPDRFSGSGSGTDFTLTISRLEPEDFAVYYCQQYGSLFTFGGGTKVEIKRTVAAPSVFIFPPSDEQLKSGTASVVCLLNNFYPREAKVQWKVDNALQSGNSQESVTEQDSKDSTYSLSSTLTLSKADYEKHKVYACEVTHQGLSSPVTKSFNRGEC

SEQ ID NO: 119 - protein, 448 aa, synthetic construct
QVQLQQWGAGLLKPSETLSLTCAVYGGSFSGYYWSWIRQTLGKGLEWIGEVSHSGGTNYNPSLKSRVTISVDTSKNQFSLKLSSVTAADTAVYYCARSPYYGDYMYVFDIWGQGTMVTVSSASTKGPSVFPLAPCSRSTSESTAALGCLVKDYFPEPVTVSWNSGALTSGVHTFPAVLQSSGLYSLSSVVTVPSSSLGTKTYTCNVDHKPSNTKVDKRVESKYGPPCPPCPAPEFLGGPSVFLFPPKPKDTLMISRTPEVTCVVVDVSQEDPEVQFNWYVDGVEVHNAKTKPREEQFNSTYRVVSVLTVLHQDWLNGKEYKCKVSNKGLPSSIEKTISKAKGQPREPQVYTLPPSQEEMTKNQVSLTCLVKGFYPSDIAVEWESNGQPENNYKTTPPVLDSDGSFFLYSRLTVDKSRWQEGNVFSCSVMHEALHNHYTQKSLSLSLGK

SEQ ID NO: 120 - protein, 450 aa, synthetic construct
EVQLLESGGGLVQPGGSLRLSCAASGFTFSSYAMSWVRQAPGKGLEWVSSISGSDFSTYYADSVKGRFTISRDTSKNTLYLQMNSLRAEDTAVYYCAKDRQWLVSSFDFWGQGALVTVSSASTKGPSVFPLAPSSKSTSGGTAALGCLVKDYFPEPVTVSWNSGALTSGVHTFPAVLQSSGLYSLSSVVTVPSSSLGTQTYICNVNHKPSNTKVDKKVEPKSCDKTHTCPPCPAPELLGGPSVFLFPPKPKDTLMISRTPEVTCVVVDVSHEDPEVKFNWYVDGVEVHNAKTKPREEQYNSTYRVVSVLTVLHQDWLNGKEYKCKVSNKALPAPIEKTISKAKGQPREPQVYTLPPSREEMTKNQVSLTCLVKGFYPSDIAVEWESNGQPENNYKTTPPVLDSDGSFFLYSKLTVDKSRWQQGNVFSCSVMHEALHNHYTQKSLSLSPGK

SEQ ID NO: 121 - protein, 447 aa, synthetic construct
EVQLLESGGGLVQPGGSLRLSCAASGFTFSSYAMSWVRQAPGKGLEWVSSISGSDFSTYYADSVKGRFTISRDTSKNTLYLQMNSLRAEDTAVYYCAKDRQWLVSSFDFWGQGALVTVSSASTKGPSVFPLAPCSRSTSESTAALGCLVKDYFPEPVTVSWNSGALTSGVHTFPAVLQSSGLYSLSSVVTVPSSSLGTKTYTCNVDHKPSNTKVDKRVESKYGPPCPPCPAPEFLGGPSVFLFPPKPKDTLMISRTPEVTCVVVDVSQEDPEVQFNWYVDGVEVHNAKTKPREEQFNSTYRVVSVLTVLHQDWLNGKEYKCKVSNKGLPSSIEKTISKAKGQPREPQVYTLPPSQEEMTKNQVSLTCLVKGFYPSDIAVEWESNGQPENNYKTTPPVLDSDGSFFLYSRLTVDKSRWQEGNVFSCSVMHEALHNHYTQKSLSLSLGK

SEQ ID NO: 122 - protein, 453 aa, synthetic construct
QVQLQESGPGLVKPSGTLSLTCAVSGGSISSSNWWSWVRQPPGKGLEWIGEVYHSGSTNYNPSLKSRVTISVDKSQNQFSLKLTSVTAADTAVYYCARVTGNKDYYYYDLDVWGQGTTVTVSSASTKGPSVFPLAPSSKSTSGGTAALGCLVKDYFPEPVTVSWNSGALTSGVHTFPAVLQSSGLYSLSSVVTVPSSSLGTQTYICNVNHKPSNTKVDKKVEPKSCDKTHTCPPCPAPELLGGPSVFLFPPKPKDTLMISRTPEVTCVVVDVSHEDPEVKFNWYVDGVEVHNAKTKPREEQYNSTYRVVSVLTVLHQDWLNGKEYKCKVSNKALPAPIEKTISKAKGQPREPQVYTLPPSREEMTKNQVSLTCLVKGFYPSDIAVEWESNGQPENNYKTTPPVLDSDGSFFLYSKLTVDKSRWQQGNVFSCSVMHEALHNHYTQKSLSLSPGK

SEQ ID NO: 123 - protein, 214 aa, synthetic construct
DIQMTQSPSSLSASVGDRVTITCQASQDISNYLNWYQQKPGKAPKLLIYDASNLGTGVPSRFSGGGSGTDFTFTISSLQPEDIATYYCQQYDNLPRTFGQGTKVEIKRTVAAPSVFIFPPSDEQLKSGTASVVCLLNNFYPREAKVQWKVDNALQSGNSQESVTEQDSKDSTYSLSSTLTLSKADYEKHKVYACEVTHQGLSSPVTKSFNRGEC

SEQ ID NO: 124 - protein, 448 aa, synthetic construct
QVQLVESGGGVVQPGRSLRLSCAASGFTFSSYGMHWVRQAPGKGLGWVAGIWYAGSNEYYVDSVKGRFIISRDNSKNTLYLQMNSLRAEDTAVYYCARDQGWGTMDAWGQGASVTVSSASTKGPSVFPLAPSSKSTSGGTAALGCLVKDYFPEPVTVSWNSGALTSGVHTFPAVLQSSGLYSLSSVVTVPSSSLGTQTYICNVNHKPSNTKVDKKVEPKSCDKTHTCPPCPAPELLGGPSVFLFPPKPKDTLMISRTPEVTCVVVDVSHEDPEVKFNWYVDGVEVHNAKTKPREEQYNSTYRVVSVLTVLHQDWLNGKEYKCKVSNKALPAPIEKTISKAKGQPREPQVYTLPPSREEMTKNQVSLTCLVKGFYPSDIAVEWESNGQPENNYKTTPPVLDSDGSFFLYSKLTVDKSRWQQGNVFSCSVMHEALHNHYTQKSLSLSPGK

SEQ ID NO: 125 - protein, 213 aa, synthetic construct
DIQMTQSPSSLSASVGDRVTITCQASQDISNYLNWYQQKPGKAPKLLIYDASNLETGVPSRFSGSGSGTDFTFTISSLQPEDIAIYYCQQYDNLLTFGGGTKVEIKRTVAAPSVFIFPPSDEQLKSGTASVVCLLNNFYPREAKVQWKVDNALQSGNSQESVTEQDSKDSTYSLSSTLTLSKADYEKHKVYACEVTHQGLSSPVTKSFNRGEC

SEQ ID NO: 126 - protein, 445 aa, synthetic construct
QVQLVESGGGVVQPGRSLRLSCAASGFTFSSYGMHWVRQAPGKGLGWVAGIWYAGSNEYYVDSVKGRFIISRDNSKNTLYLQMNSLRAEDTAVYYCARDQGWGTMDAWGQGASVTVSSASTKGPSVFPLAPCSRSTSESTAALGCLVKDYFPEPVTVSWNSGALTSGVHTFPAVLQSSGLYSLSSVVTVPSSSLGTKTYTCNVDHKPSNTKVDKRVESKYGPPCPPCPAPEFLGGPSVFLFPPKPKDTLMISRTPEVTCVVVDVSQEDPEVQFNWYVDGVEVHNAKTKPREEQFNSTYRVVSVLTVLHQDWLNGKEYKCKVSNKGLPSSIEKTISKAKGQPREPQVYTLPPSQEEMTKNQVSLTCLVKGFYPSDIAVEWESNGQPENNYKTTPPVLDSDGSFFLYSRLTVDKSRWQEGNVFSCSVMHEALHNHYTQKSLSLSLGK

SEQ ID NO: 127 - protein, 598 aa, synthetic construct
MTPIVTVLICLGLSLGPRTHVQTGTIPKPTLWAEPDSVITQGSPVTLSCQGSLEAQEYRLYREKKSASWITRIRPELVKNGQFHIPSITWEHTGRYGCQYYSRARWSELSDPLVLVMTGAYPKPTLSAQPSPVVTSGGRVTLQCESQVAFGGFILCKEGEEEHPQCLNSQPHARGSSRAIFSVGPVSPNRRWSHRCYGYDLNSPYVWSSPSDLLELLVPGVSKKPSLSVQPGPVVAPGESLTLQCVSDVGYDRFVLYKEGERDLRQLPGRQPQAGLSQANFTLGPVSRSYGGQYRCYGAHNLSSECSAPSDPLDILITGQIRGTPFISVQPGPTVASGENVTLLCQSWRQFHTFLLTKAGAADAPLRLRSIHEYPKYQAEFPMSPVTSAHAGTYRCYGSLNSDPYLLSHPSEPLELVVSGPSMGSSPPPTGPISTPAGPEDQPLTPTGSDPQSGLGRHLGVVIGILVAVVLLLLLLLLLFLILRHRRQGKHWTSTQRKADFQHPAGAVGPEPTDRGLQWRSSPAADAQEENLYAAVKDTQPEDGVEMDTRAAASEAPQDVTYAQLHSLTLRRKATEPPPSQEREPPAEPSIYATLAIH

SEQ ID NO: 128 - protein, 605 aa, synthetic construct
MTPILTILICLGLSLGSRTHVQAGTLPKPTLWAEPGSMISEGSPVTLRCQGNLQVQDYRLQREKKPASWVRQIRQELVKKGYFAIASITWEHTGRYRCQYYSHSCWSEPSDPLELVVIGAYSKPTLSALPSPVVASGGNVTLQCDSQVAFDGFILCKEGEDEHPQRLNSQSHVHGWSWAVFSVGPVSPSHRWSYRCYGYISSAPYVWSLPSDLLELLVPGVSKKPSLSVQPGPVVARGDKLTLQCGSGAGYDRFALYKEGERDFLQRPGQQLQAGLSQANFLLGPVRGSHGGQYRCYGAHNLSPEWSAPSDPLDILISRQIRGTPFLSVQPGPKVVSGENVTLLCQSSWQFHAFLLTQAGAADAHLHLRSMHKYPKYQAEFPISPVTSAHAGTYRCYGSRSSNPYLLSVPSDPLELVVSGPSGGPSSPTTGPTSPTTGPTSTCAGPEDQPLTPTGSDSQSGLGRHLGVVTGILVAFVLLLFLLLLLFLVLRHRRQGKRWTSAQRKADFQHPAGAVEPEPRDRGLQRRSSPAANTQEENLYAAVKDTQPEDGVELDSRAAASEDPQDVTYAQLQSLTLRRETTEPPPSQERAPPVESSIYATLTIH

SEQ ID NO: 129 - protein, 650 aa, synthetic construct
MTPILTVLICLGLSLGPRTHVQAGHLPKPTLWAEPGSVITQGSPVTLRCQGGQETQEYRLYREKKTALWITRIPQELVKKGQFPIPSITWEHAGRYRCYYGSDTAGRSESSDPLELVVTGAYIKPTLSAQPSPVVNSGGNVILQCDSQVAFDGFSLCKEGEDEHPQCLNSQPHARGSSRAIFSVGPVSPSRRWWYRCYAYDSNSPYEWSLPSDLLELLVLGVSKKPSLSVQPGPIVAPEETLTLQCGSDAGYNRFVLYKDGERDFLQLAGAQPQAGLSQANFTLGPVSRSYGGQYRCYGAHNLSSEWSAPSDPLDILIAGQFYDRVSLSVQPGPTVASGENVTLLCQSQGWMQTFLLTKEGAADDPWRLRSTYQSQKYQAEFPMGPVTSAHAGTYRCYGSQSSKPYLLTHPSDPLELVVSGPSGGPSSPTTGPTSTSGPEDQPLTPTGSDPQSGLGRHLGVVIGILVAVILLLLLLLLLFLILRHRRQGKHWTSTQRKADFQHPAGAVGPEPTDRGLQWRSSPAADAQEENLYAAVKHTQPEDGVEMDTRSPHDEDPQAVTYAEVKHSRPRREMASPPSPLSGEFLDTKDRQAEEDRQMDTEAAASEAPQDVTYAQLHSLTLRREATEPPPSQEGPSPAVPSIYATLAIH

SEQ ID NO: 130 - protein, 761 aa, synthetic construct
MALPALGLDPWSLLGLFLFQLLQLLLPTTTAGGGGQGPMPRVRYYAGDERRALSFFHQKGLQDFDTLLLSGDGNTLYVGAREAILALDIQDPGVPRLKNMIPWPASDRKKSECAFKKKSNETQCFNFIRVLVSYNVTHLYTCGTFAFSPACTFIELQDSYLLPISEDKVMEGKGQSPFDPAHKHTAVLVDGMLYSGTMNNFLGSEPILMRTLGSQPVLKTDNFLRWLHHDASFVAAIPSTQVVYFFFEETASEFDFFERLHTSRVARVCKNDVGGEKLLQKKWTTFLKAQLLCTQPGQLPFNVIRHAVLLPADSPTAPHIYAVFTSQWQVGGTRSSAVCAFSLLDIERVFKGKYKELNKETSRWTTYRGPETNPRPGSCSVGPSSDKALTFMKDHFLMDEQVVGTPLLVKSGVEYTRLAVETAQGLDGHSHLVMYLGTTTGSLHKAVVSGDSSAHLVEEIQLFPDPEPVRNLQLAPTQGAVFVGFSGGVWRVPRANCSVYESCVDCVLARDPHCAWDPESRTCCLLSAPNLNSWKQDMERGNPEWACASGPMSRSLRPQSRPQIIKEVLAVPNSILELPCPHLSALASYYWSHGPAAVPEASSTVYNGSLLLIVQDGVGGLYQCWATENGFSYPVISYWVDSQDQTLALDPELAGIPREHVKVPLTRVSGGAALAAQQSYWPHFVTVTVLFALVLSGALIILVASPLRALRARGKVQGCETLRPGEKAPLSREQHLQSPKECRTSASDVDADNNCLGTEVA

SEQ ID NO: 131 - protein, 338 aa, synthetic construct
MVVMAPRTLFLLLSGALTLTETWAGSHSMRYFSAAVSRPGRGEPRFIAMGYVDDTQFVRFDSDSACPRMEPRAPWVEQEGPEYWEEETRNTKAHAQTDRMNLQTLRGYYNQSEASSHTLQWMIGCDLGSDGRLLRGYEQYAYDGKDYLALNEDLRSWTAADTAAQISKRKCEAANVAEQRRAYLEGTCVEWLHRYLENGKEMLQRADPPKTHVTHHPVFDYEATLRCWALGFYPAEIILTWQRDGEDQTQDVELVETRPAGDGTFQKWAAVVVPSGEEQRYTCHVQHEGLPEPLMLRWKQSSLPTIPIMGIVAGLVVLAAVVTGAAVAAVLWRKKSSD

SEQ ID NO: 132 - protein, 119 aa, synthetic construct
MSRSVALAVLALLSLSGLEAIQRTPKIQVYSRHPAENGKSNFLNCYVSGFHPSDIEVDLLKNGERIEKVEHSDLSFSKDWSFYLLYYTEFTPTEKDEYACRVNHVTLSQPKIVKWDRDM

SEQ ID NO: 133 - protein, 121 aa, synthetic construct
EVQLQQWGAGLLKPSETLSLTCAVYGGSFSGYYWSWIRQPPGKGLEWIGEINHAGSTNYNPSLKSRVTISVDTSKNQFSLKLSSVTAADTAVYYCARLPTRWVTTRYFDLWGRGTLVTVSS

SEQ ID NO: 134 - protein, 111 aa, synthetic construct
ESVLTQPPSVSGAPGQRVTISCTGSSSNIGAGYDVHWYQQLPGTAPKLLIYGDSNRPSGVPDRFSVSKSGASASLAITGLQAEDEADYYCQSFDNSLSAYVFGGGTQLTVL

SEQ ID NO: 135 - protein, 125 aa, synthetic construct
EVQLLESGGGLVQPGGSLRLSCAASGFTFSNYAMNWVRQAPGKGLEWVSVISVSGGSTYYADSVKGRFTISRDNSKNTLYLQMNSLRAEDTAVYYCAKDYYYDSGSYYDSFFDYWGQGTLVTVSS

SEQ ID NO: 136 - protein, 108 aa, synthetic construct
EIVLTQSPGTLSLSPGERATLSCRASQSVSSSYLAWYQQKPGQAPRLLIYGASSRATGIPDRFSGSGSGTDFTLTISRLEPEDFAVYYCQQYGSSPLTFGGGTKVEIK

SEQ ID NO: 137 - protein, 125 aa, synthetic construct
QVQLVQSGAEVKKPGASVKVSCKASGYTFTDYYINWVRQAPGQGLEWMGNVNPNDGGTTYNQKFKGRVTMTTDTSTSTAYMELRSLRSDDTAVYYCARREIYFYGTIYYYAMDYWGQGTLVTVSS

SEQ ID NO: 138 - protein, 111 aa, synthetic construct
DIQLTQSPSFLSASVGDRVTITCRASESVDYYGNSFMYWYQQKPGKAPKLLIYFASNLESGVPSRFSGSGSGTEFTLTISSLQPEDFATYYCQQNNEDPWTFGGGTKVEIK